European Patent Specification EP 4 047 007 B1, published June 5, 2024. Title: PEPTIDE AND USE THEREOF IN TREATING INFLAMMATORY DISEASE AND PAIN. Applicant: PELL BIO-MED TECHNOLOGY CO., LTD. The sequence listing filed with the application follows.

SEQUENCE LISTING (1 sequence)

SEQ ID NO: 1 - protein, 11 aa, Artificial Sequence
  MOD_RES (1)..(1): PYRROLIDONE CARBOXYLIC ACID
XETAVSSHEQD